European Patent Application EP 4 786 584 A1, published August 5, 2026. Title: 用于单分子测序的核酸聚合酶及其突变株. Applicant: 成都今是科技有限公司. The sequence listing filed with the application follows.

SEQUENCE LISTING (40 sequences)

SEQ ID NO: 1 - protein, 566 aa, Actinomyces naeslundii
MVRQSTIASPARGGVRRSHKKVPSFCADFETTTDEDDCRVWSWGIIQVGKLQNYVDGISLDGFMSHISERASHIYFHNLAFDGTFILDWLLKHGYRWTKENPGVKEFTSLISRMGKYYSITVVFETGFRVEFRDSFKKLPMSVSAIAKAFNLHDQKLEIDYEKPRPIGYIPTEQEKRYQRNDVAIVAQALEVQFAEKMTKLTAGSDSLATYKKMTGKLFIRRFPILSPEIDTEIRKAYRGGFTYADPRYAKKLNGKGSVYDVNSLYPSVMRTALLPYGEPIYSEGAPRTNRPLYIASITFTAKLKPNHIPCIQIKKNLSFNPTQYLEEVKEPTTVVATNIDIELWKKHYDFKIYSWNGTFEFRGSHGFFDTYVDHFMEIKKNSTGGLRQIAKLHLNSLYGKFATNPDITGKHPTLKDNRVSLVMNEPETRDPVYTPMGVFITAYARKKTISAAQDNYETFAYADTDSLHLIGPTTPPDSLWVDPVELGAWKHESSFTKSVYIRAKQYAEEIGGKLDVHIAGMPRNVAATLTLEDMLHGGTWNGKLIPVRVPGGTVLKDTTFTLKID

SEQ ID NO: 2 - protein, 566 aa, synthetic construct
  source 1..566: organism (original language) = 合成构建体
MVRQSTIASPARGGVRRSHKKVPSFCADFETTTDEDDCRVWSWGIIQVGKLQNYVDGISLDGFMSHISERASHIYFHNLAFDGTFILDWLLKHGYRWTKENPGVKEFTSLISRMGKYYSITVVFETGFRVEFRDSFKKLPMSVSAIAKAFNLHDQKLEIDYEKPRPIGYIPTEQEKRYQRNDVAIVAQALEVQFAEKATKLTAGSDSLATYKKMTGKLFIRRFPILSPEIDTEIRKAYRGGFTYADPRYAKKLNGKGSVYDVQSLYPSVMRTALLPYGEPIYSEGAPRTNRPLYIASITFTAKLKPNHIPCIQIKKNLSFNPTQYLEEVKEPTTVVATNIDIELWKKHYDFKIYSWNGTFEFRGSHGFFDTYVDHFMQIKKNSTGGLRQIAKLHLNSLYGKFATNPDITGKHPTLKDNRVSLVMNEPETRDPVYTPMGVFITAYARKKTISAAQDNYETIAYADTDSLHLIGPTTPPDSLWVDPVELGAWKHESSFTKSVYIRAKQYAEEIGGKLDVRIAGMPRNVAATLTLEDMLHGGTWNGKLIPVRVPGGTVLKDTTFTLKID

SEQ ID NO: 3 - protein, 566 aa, synthetic construct
  source 1..566: organism (original language) = 合成构建体
MVRQSTIASPARGGVRRSHKKVPSFCADFETTTDEDDCRVWSWGIIQVGKLQNYVDGISLDGFMSHISERASHIYFHNLAFDGTFILDWLLKHGYRWTKENPGVKEFTSLISRMGKYYSITVVFETGFRVEFRDSFKKLPMSVSAIAKAFNLHDQKLEIDYEKPRPIGYIPTEQEKRYQRNDVAIVAQALEVQFAEKATKLTAGSDSLATYKKMTGKLFIRRFPILSPEIDTEIRKAYRGGFTYADPRYAKKLNGKGSVYDVQSLYPSVMRTALLPYGEPIYSEGAPRTNRPLYIASITFTAKLKPNHIPCIQIKKNLSFNPTQYLEEVKEPTTVVATNIDIELWKKHYDFKIYSWNGTFEFRGSHGFFDTSVDHFMEIKKNSKGGLRQIAKLHLNSLYGKFATNPDITGKHPTLKDNRVSLVMNEPETRDPVYTPMGVFITAYARKKTISAAQDNYETFAYADTDSLHLIGPTTPPDSLWVDPVELGAWKHESSFTKSVYIRAKQYAEEIGGKLDVHIAGMPRNVAATLTLEDMLHGGTWNGKLIPVRVPGGTVLKDTTFTLKID

SEQ ID NO: 4 - protein, 566 aa, synthetic construct
  source 1..566: organism (original language) = 合成构建体
MVRQSTIASPARGGVRRSHKKVPSFCADFETTTDEDDCRVWSWQIIQVGKLQNYVDGISLDGFMSHISERASHIYFHNLAFDGTFILDWLLKHGYRWTKENPGVKEFTSLISRMGKYYSITVVFETGFRVEFRDSFKKLPMSVSAIAKAFNLHDQKLEIDYEKPRPIGYIPTEQEKRYQRNDVAIVAQALEVQFAEKATKLTAGSDSLATYKKMTGKLFIRRFPILSPEIDTEIRKAYRGGFTYADPRYAKKLNGKGSVYDVNSLYPSVMRTALLPYGEPIYSEGAPRTNRPLYIASITFTAKLKPNHIPCIQIKKNLSFNPTQYLEEVKEPTTVVATNIDIELWKKHYDFKIYSWNGTFEFRGSHGFFDTSVDHFMEIKKNSKGGLRQIAKLHLNSLYGKFATNPDITGKHPTLKDNRVSLVMNEPETRDPVYTPMGVFITAYARKKTISAAQDNYETFAYADTDSLHLIGPTTPPDSLWVDPVELGAWRHESSFTKSVYIRAKQYAEEIGGKLDVHIAGMPRNVAATLTLEDMLHGGTWNGKLIPVRVPGGTVLKDTTFTLKID

SEQ ID NO: 5 - protein, 566 aa, synthetic construct
  source 1..566: organism (original language) = 合成构建体
MVRQSTIASPARGGVRRSHKKVPSFCADFETTTDEDDCRVWSWGIIQVGKLQNYVDGISLDGFMSHISERASHIYFHNLAVDGTFILDWLLKHGYRWTKENPGVKEFTSLISRMGKYYSITVVFETGFRVEFRDSFKKLPMSVSAIAKAFNLHDQKLEIDYEKPRPIGYIPTEQEKRYQRNDVAIVAQALEVQFAEKATKLTAGSDSLATYKKMTGKLFIRRFPILSPEIDTEIRKAYRGGFTYADPRYAKKLNGKGSVYDVNSLYPSVMRTALLPYGEPIYSEGAPRTNRPLYIASITFTAKLKPNHIPCIQIKKNNSFNPTQYLEEVKEPTTVVATNIDIELWKKHYDFKIYSWNGTFEFRGSHGFFDTYVDHFMQIKKNSKGGLRQIAKLHLNSLYGKFATNPDITGKHPTLKDNRVSLVMNEPETRDPVYTPMGVFITAYARKKTISAAQDNYETFAYADTDSLHLIGPTTPPDSLWVDPVELGAWKHESSFTKSVYIRAKQYAEEIGGKLDVHIAGMPRNVAATLTLEDMLHGGTWNGKLIPVRVPGGTVLKDTTFTLKID

SEQ ID NO: 6 - protein, 566 aa, synthetic construct
  source 1..566: organism (original language) = 合成构建体
MVRQSTIASPARGGVRRSHKKVPSFCADFATTTDEDDCRVWSWGIIQVGKLQNYVDGISLDGFMSHISERASHIYFHNLAFDGTFILDWLLKHGYRWTKENPGVKEFTSLISRMGKYYSITVVFETGFRVEFRDSFKKLPMSVSAIAKAFNLHDQKLEIDYEKPRPIGYIPTEQEKRYQRNDVAIVAQALEVQFAEKMTKLTAGSDSLATYKKMTGKLFIRRFPILSPEIDTEIRKAYRGGFTYADPRYAKKLNGKGSVYDVNSLYPSVMRTALLPYGEPIYSEGAPRTNRPLYIASITFTAKLKPNHIPCIQIKKNNSFNPTQYLEEVKEPTTVVATNIDIELWKKHYDFKIYSWNGTFEFRGSHGFFDTYVDHFMQIKKNSKGGLRRIAKLHLNSLYGKFATNPDITGKHPTLKDNRVSLVMNEPETRDPVYTPMGVFITAYARKKTISAAQDNYETFAYADTDSLHLIGPTTPPDSLWVDPVELGAWKHESSFTKSVYIRAKQYAEEIGGKLDVHIAGMPRNVAATLTLEDMLHGGTWNGKLIPVRVPGGTVLKDTTFTLKID

SEQ ID NO: 7 - protein, 566 aa, synthetic construct
  source 1..566: organism (original language) = 合成构建体
MVRQSTIASPARGGVRRSHKKVPSFCADFETTTDEDDCRVWSWGIIQVGKLQNYVDGISLDGFMSHISERASHIYFHNLAFDGTFILDWLLKHGYRWTKENPGVKEFTSLISRVGKYYSITVVFETGFRVEFRDSFKKLPMSVSAIAKAFNLHDQKLEIDYEKPRPIGYIPTEQEKRYQRNDVAIVAQALEVQFAEKMTKLTAGSDSLATYKKMTGKLFIRRFPILSPEIDTEIRKAYRGGFTYADPRYAKKLNGKGSVYDVNSAYPSVMRTALLPYGEPIYSEGAPRTNRPLYIASITFTAKLKPNHIPCIQIKKNLSFNPTQYLEEVKEPTTVVATNIDIELWKKHYDFKIYSWNGTFEFRGSHGFFDTYVDHFMEIKKNSKGGLRQIAKLHLNSLYGKFATNPDITGKHPTLKDNRVSLVMNEPETRDPVYTPMGVFIKAYARKKTISAAQDNYETFAYADTDSLHLIGPTTPPDSLWVDPVELGAWKHESSFTKSVYIRAKQYAEEIQGKLDVHIAGMPRNVAATLTLEDMLHGGTWNGKLIPVRVPGGTVLKDTTFTLKID

SEQ ID NO: 8 - protein, 566 aa, synthetic construct
  source 1..566: organism (original language) = 合成构建体
MVRQSTIASPARGGVRRSHKKVPSFCADFETTTDEDDCRVWSWGIIQVGKLQNYVDGISLDGFMSHISERASHIYFHNLAFDGTFILDWLLKHGYRWTKENPGVKEFTSLISRMGKYYSITVVFETGFRVEFRDSFKKLPMSVSAIAKAFNLHDQKLEIDYEKPRPIGYIPTEQEKRYQRNDVAIVAQALEVQFAEKMTKLTAGSDSLATYKKMTGKLFIRRFPILSPEIDTEIRKAYRGGFTYADPRYAKKLNGKGSVYDVNSLYPSVMRTKLLPYGEPIYSEGAPRTNRPLYIASITFTAKLKPNHIPCIQIKKRLSFNPTQYLEEVKEPTTVVATNIDIELWKKHYDFKIYSWNGTFEFRGSHGFFDTYVDHFMQKKKNSTGGLRQIAKLHLNSLYGKFATNPDITGKHPTLKDNRVSLVMNEPETRDPVYTPMGVFITAYARKKTISAAQDNYETFAYADTDSLHLIGPTTPPDSLWVDPVELGAWRHESSFTKSVYIRAKQYAEEIGGKLDVHIAGMPRNVAATLTLEDMLHGGTWNGKLIPVRVPGGTVLKDTTFTLKID

SEQ ID NO: 9 - protein, 566 aa, synthetic construct
  source 1..566: organism (original language) = 合成构建体
MVRQSTIASPARGGVRRSHKKVPSFCADFETTTDEDDCRVWSWGIIQVGKLQNYVDGISLDGFMSHISERASHIYFHNLAFDGTFILDWLLKHGYRWTKENPGVKEFTSLISRMGKYYSITVVFETGFRVEFRDSFKKLPMSVSAIAKAFNLHDQKLEIDYEKPRPIGYIPTEQEKRYQRNDVAIVAQALEVQFAEKMTKLTAGSDSLATYKKMTGKLFIRRFPILSPEIDTEIRKAYRGGFTYADPRYAKKLNGKGSVYDVNSLYPSVMRTKLLPYGEPIYSEGAPRTNRPLYIASITFTAKLKPNHIPCIQIKKRLSFNPTQYLEEVKEPTTVVATNIDIELWKKHYDFKIYSWNGTFEFRGSHGFFDTYVDHFMQKKKNSTGGLRQIAKLHLNSLYGKFATNPDITGKHPTLKDNRVSLVMNEPETRDPVYTPMGVFITAYARKKTISAAQDNYETFAYADTDSLHLIGPTTPPDSLWVDPVELGAWKHKSSFTKSVYIRAKQYAEEIGGKLDVHIAGMPRNVAATLTLEDMLHGGTWNGKLIPVRVPGGTVLKDTTFTLKID

SEQ ID NO: 10 - protein, 566 aa, synthetic construct
  source 1..566: organism (original language) = 合成构建体
MVRQSTIASPARGGVRRSHKKVPSFCADFATTTDEDDCRVWSWGIIQVGKLQNYVDGISLDGFMSHISERASHIYFHNLAFDGTFILDWLLKHGYRWTKENPGVKEFTSLISRMGKYYSITVVFETGFRVEFRDSFKKLPMSVSAIAKAFNLHDQKLEIDYEKPRPIGYIPTEQEKRYQRNDVAIVAQALEVQFAEKMTKLTAGSDSLATYKKMTGKLFIRRFPILSPEIDTEIRKAYRGGFTYADPRYAKKLNGKGSVYDVNSAYPSVMRTALLPYGEPIYSEGAPRTNRPLYIASITFTAKLKPNHIPCICIKKNLSFNPTQYLEEVKEPTTVVATNIDIELWKKHYDFKIYSWNGTFEFRGSHGFFDTYVDHFMEIKKNSTGGLRQIAKLILNSLYGKFATNPDITGKHPTLKDNRVSLVMNEPETRDPVYTPMGVFITAYARKKTISAAQDNYETFAYADTDSLHLIGPTTPPDSLWVDPVELGAWMHESSFTKSVYIRAKQYAEEIGGKLDVHIAGMPRNVAATLTLEDMLHGGTWNGKLIPVRVPGGTVLKDTTFTLKID

SEQ ID NO: 11 - protein, 566 aa, synthetic construct
  source 1..566: organism (original language) = 合成构建体
MVRQSTIASPARGGVRRSHKKVPSFCADFETTTDEDDCRVWSWGIIQVGKLQNYVDGISLDGFMSHISERASHIYFHNLAIDGTFILDWLLKHGYRWTKENPGVKEFTSLISRMGKYYSITVVFETGFRVEFRDSFKKLPMSVSAIAKAFNLHDQKLEIDYEKPRPIGYIPTEQEKRYQRNDVAIVAQALEVQFAEKMTKLTAGSDSLATYKKMTGKLFIRRFPILSPEIDTEIRKAYRGGFTYADPRYAKKLNGKGSVYDVNSAYPSVMRTALLPYGEPIYSEGAPRTNRPLYIASITFTAKLKPNHIPCIQIKKNLSFNPTQYLEEVKEPTTVVATNIDIELWKKHYDFKIYSWNGTFEFRGSHGFFDTYVDHFMQIKKNSKGGLRQIAKLHLNSLYGKFATNPDITGKHPTLKDNRVSLVMNEPETRDPVYTPMGVFITAYARKKTISAAQDNYETFAYADTDSLHLIGPTTPPDSLWVDPVELGAWRHKSSFTKSVYIRAKQYAEEIGGKLDVHIAGMPRNVAATLTLEDMLHGGTWNGKLIPVRVPGGTVLKDTTFTLKID

SEQ ID NO: 12 - protein, 566 aa, synthetic construct
  source 1..566: organism (original language) = 合成构建体
MVRQSTIASPARGGVRRSHKKVPSFCADFETTTDEDDCRVWSWGIIQVGKLQNYVDGISLDGFMSHISERASHIYFHNLAVDGTFILDWLLKHGYRWTKENPGVKEFTSLISRMGKYYSITVVFETGFRVEFRDSFKKLPMSVSAIAKAFNLHDQKLEIDYEKPRPIGYIPTEQEKRYQRNDVAIVAQALEVQFAEKMTKLTAGSDSLATYKKMTGKLFIRRFPILSPEIDTEIRKAYRGGFTYADPRYAKKLNGKGSVYDVNSAYPSVMRTALLPYGEPIYSEGAPRTNRPLYIASITFTAKLKPNHIPCIQIKKNLSFNPTQYLEEVKEPTTVVATNIDIELWKKHYDFKIYSWNGTFEFRGSHGFFDTYVDHFMQIKKNSKGGLRQIAKLHLNSLYGKFATNPDITGKHPTLKDNRVSLVMNEPETRDPVYTPMGVFITAYARKKTISAAQDNYETFAYADTDSLHLIGPTTPPDSLWVDPVELGAWRHKSSFTKSVYIRAKQYAEEIGGKLDVHIAGMPRNVAATLTLEDMLHGGTWNGKLIPVRVPGGTVLKDTTFTLKID

SEQ ID NO: 13 - protein, 566 aa, synthetic construct
  source 1..566: organism (original language) = 合成构建体
MVRQSTIASPARGGVRRSHKKVPSFCADFATTTDEDDCRVWSWGIIQVGKLQNYVDGISLDGFMSHISERASHIYFHNLAFDGTFILDWLLKHGYRWTKENPGVKEFTSLISRMGKYYSITVVFETGFRVEFRDSFKKLPMSVSAIAKAFNLHDQKLEIDYEKPRPIGYIPTEQEKRYQRNDVAIVAQALEVQFAEKMTKLTAGSDSLATYKKMTGKLFIRRFPILSPEIDTEIRKAYRGGFTYADPRYAKKLNGKGSVYDVNSIYPSVMRTALLPYGEPIYSEGAPRTNRPLYIASITFTAKLKPNHIPCICIKKNLSFNPTQYLEEVKEPTTVVATNIDIELWKKHYDFKIYSWNGTFEFRGSHGFFDTYVDHFMEIKKNSTGGLRQIAKLILNSLYGKFATNPDITGKHPTLKDNRVSLVMNEPETRDPVYTPMGVFITAYARKKTISAAQDNYETFAYADTDSLHLIGPTTPPDSLWVDPVELGAWMHESSFTKSVYIRAKQYAEEIGGKLDVHIAGMPRNVAATLTLEDMLHGGTWNGKLIPVRVPGGTVLKDTTFTLKID

SEQ ID NO: 14 - protein, 566 aa, synthetic construct
  source 1..566: organism (original language) = 合成构建体
MVRQSTIASPARGGVRRSHKKVPSFCADFATTTDEDDCRVWSWGIIQVGKLQNYVDGISLDGFMSHISERASHIYFHNLAFDGTFILDWLLKHGYRWTKENPGVKEFTSLISRMGKYYSITVVFETGFRVEFRDSFKKLPMSVSAIAKAFNLHDQKLEIDYEKPRPIGYIPTEQEKRYQRNDVAIVAQALEVQFAEKMTKLTAGSDSLATYKKMTGKLFIRRFPILSPEIDTEIRKAYRGGFTYADPRYAKKLNGKGSVYDVNSVYPSVMRTALLPYGEPIYSEGAPRTNRPLYIASITFTAKLKPNHIPCICIKKNLSFNPTQYLEEVKEPTTVVATNIDIELWKKHYDFKIYSWNGTFEFRGSHGFFDTYVDHFMEIKKNSTGGLRQIAKLILNSLYGKFATNPDITGKHPTLKDNRVSLVMNEPETRDPVYTPMGVFITAYARKKTISAAQDNYETFAYADTDSLHLIGPTTPPDSLWVDPVELGAWKHVSSFTKSVYIRAKQYAEEIGGKLDVHIAGMPRNVAATLTLEDMLHGGTWNGKLIPVRVPGGTVLKDTTFTLKID

SEQ ID NO: 15 - protein, 566 aa, synthetic construct
  source 1..566: organism (original language) = 合成构建体
MVRQSTIASPARGGVRRSHKKVPSFCADFETTTDEDDCRVWSWGIIQVGKLQNYVDGISLDGFMSHISERASHIYFHNLAFDGTFILDWLLKHGYRWTKENPGVKEFTSLISRMGKYYSITVVFETGFRVEFRDSFKKLPMSVSAIAKAFNLHDQKLEIDYEKPRPIGYIPTEQEKRYQRNDVAIVAQALEVQFAEKMTKLTAGSDSLATYKKMTGKLYIRRFPILSPEIDTEIRKAYRGGFTYADPRYAKKLNGKGSVYDVNSIYPSVMRTALLPYGEPIYSEGAPRTNRPLYIASITFTAKLKPNHIPCIQIKKNLSFNPTQYLEEVREPTTVVATNIDIELWKKHYDFKIYSWNGTFEFRGSHGFFDTYVDHFMEIKKNSTGGLRQIAKLHLNSLYGKFATNPDITGKHPTLKDNRVSLVMNEPETRDPVYTPMGVFITAYARKKTISAAQDNYETFAYADTDSLHLIGPTTPPDSLWVDPVELGAWRHESSFTKSVYLRAKQYAEEIGGKLDVHIAGMPRNVAATLTLEDMLHGGTWNGKLIPVRVPGGTVLKDTTFTLKID

SEQ ID NO: 16 - protein, 566 aa, synthetic construct
  source 1..566: organism (original language) = 合成构建体
MVRQSTIASPARGGVRRSHKKVPSFCADFETTTDEDDCRVWSWGIIQVGKLQNYVDGISLDGFMSHISERASHIYFHNLAVDGTFILDWLLKHGYRWTKENPGVKEFTSLISRMGKYYSITVVFETGFRVEFRDSFKKLPMSVSAIAKAFNLHDQKLEIDYEKPRPIGYIPTEQEKRYQRNDVAIVAQALEVQFAEKMTKLTAGSDSLATYKKMTGKLYIRRFPILSPEIDTEIRKAYRGGFTYADPRYAKKLNGKGSVYDVNSIYPSVMRTALLPYGEPIYSEGAPRTNRPLYIASITFTAKLKPNHIPCIQIKKNLSFNPTQYLEEVKEPTTVVATNIDIELWKKHYDFKIYSWNGTFEFRGSHGFFDTYVDHFMEIKKNSKGGLRQIAKLHLNSLYGKFATNPDITGKHPTLKDNRVSLVMNEPETRDPVYTPMGVFITAYARKKTISAAQDNYETFAYADTDSLHLIGPTTPPDSLWVDPVELGAWKHESSFTKSVYLRAKQYAEEIGGKLDVHIAGMPRNVAATLTLEDMLHGGTWNGKLIPVRVPGGTVLKDTTFTLKID

SEQ ID NO: 17 - protein, 566 aa, synthetic construct
  source 1..566: organism (original language) = 合成构建体
MVRQSTIASPARGGVRRSHKKVPSFCADFETTTDEDDCRVWSWGIIQVGKLQNYVDGISLDGFMSHISERASHIYFHNLAFDGTFILDWLLKHGYRWTKENPGVKEFTSLISRMGKYYSITVVFETGFRVEFRDSFKKLPMSVSAIAKAFNLHDQKLEIDYEKPRPIGYIPTEQEKRYQRNDVAIVAQALEVQFAEKMTKLTAGSDSLATYKKMTGKLFIRRFPILSPEIDTEIRKAYRGGFTYADPRYAKKLNGKGSVYDVNSAYPSVMRTALLPYGEPIYSEGAPRTNRPLYIASITFTAKLKPNHIPCIQIKKNLSFNPTQYLEEVKEPTTVVATNIDIELWKKHYDFKIYSWNGTFEFRGSHGFFDTYVDHFMQIKKNSKGGLRQIAKLHLNSLYGKFATNPDITGKHPTLKDNRVSLVMNEPETRDPVYTPMGVFITAYARKKTISAAQDNYETFAYADTDSLHLIGPTTPPDSLWVDPVELGAWRHKSSFTKSVYIRAKQYAEEIGGKLDVHIAGMPRNVAATLTLEDMLHGGTWNGKLIPVRVPGGTVLKDTTFTLKID

SEQ ID NO: 18 - protein, 566 aa, synthetic construct
  source 1..566: organism (original language) = 合成构建体
MVRQSTIASPARGGVRRSHKKVPSFCADFETTTDEDDCRVWSWGIIQVGKLQNYVDGISLDGFMSHISERASHIYFHNLAFDGTFILDWLLKHGYRWTKENPGVKEFTSLISRMGKYYSITVVFETGFRVEFRDSFKKLPMSVSAIAKAFNLHDQKLEIDYEKPRPIGYIPTEQEKRYQRNDVAIVAQALEVQFAEKMTKLTAGSDSLATYKKMTGKLYIRRFPILSPEIDTEIRKAYRGGFTYADPRYAKKLNGKGSVYDVNSLYPSVMRSALLPYGEPIYSEGAPRTNRPLYIASITFTAKLKPNHIPCIQIKKNNSFNPTQYLEEVKEPTTVVATNIDIELWKKHYDFKIYSWNGTFEFRGSHGFFDTYVDHFMQIKKNSTGGLRQIAKLHLNSLYGKFATNPDITGKHPTLKDNRVSLVMNEPETRDPVYTPMGVFITAYARKKTISAAQDNYETFAYADTDSLHLIGPTTPPDSLWVDPVELGAWKHESSFTKSVYIRAKQYAEEIGGKLRVHIAGMPRNVAATLTLEDMLHGGTWNGKLIPVRVPGGTVLKDTTFTLKID

SEQ ID NO: 19 - protein, 566 aa, synthetic construct
  source 1..566: organism (original language) = 合成构建体
MVRQSTIASPARGGVRRSHKKVPSFCADFETTTDEDDCRVWSWQIIQVGKLQNYVDGISLDGFMSHISERASHIYFHNLAFDGTFILDWLLKHGYRWTKENPGVKEFTSLISRMGKYYSITVVFETGFRVEFRDSFKKLPMSVSAIAKAFNLHDQKLEIDYEKPRPIGYIPTEQEKRYQRNDVAIVAQALEVQFAEKMTKLTAGSDSLATYKKMTGKLFIRRFPILSPEIDTEIRKAYRGGFTYADPRYAKKLNGKGSVYDVNSLYPSVMRSALLPYGEPIYSEGAPRTNRPLYIASITFTAKLKPNHIPCIQIKKNLSFNPTQYLEEVKEPTTVVATNIDIELWKKHYDFKIYSWNGTFEFRGSHGFFDTYVDHFMDIKKNSTGGLRQIAKLHLNSLYGKFATNPDITGKHPTLKDNRVSLVMNEPETRDPVYTPMGVFITAYARKKTISAAQDNYETFAYADTDSLHLIGPTTPPDSLWVDPVELGAWKHKSSFTKSVYIRAKQYAEEIQGKLDVHIAGMPRNVAATLTLEDMLHGGTWNGKLIPVRVPGGTVLKDTTFTLKID

SEQ ID NO: 20 - protein, 566 aa, synthetic construct
  source 1..566: organism (original language) = 合成构建体
MVRQSTIASPARGGVRRSHKKVPSFCAQFETTTDEDDCRVWSWGIIQVGKLQNYVDGISLDGFMSHISERASHIYFHNLAFDGTFILDWLLKHGYRWTKENPGVKEFTSLISRMGKYYSITVVFETGFRVEFRDSFKKLPMSVSAIAKAFNLHDQKLEIDYEKPRPIGYIPTEQEKRYQRNDVAIVAQALEVQFAEKMTKLTAGSDSLATYKKMTGKLFIRRFPILSPEIDTEIRKAYRGGFTYADPRYAKKLNGKGSVYDVNSLYPSVMRYALLPYGEPIYSEGAPRTNRPLYIASITFTAKLKPNHIPCIQIKKNLSFNPTQYLEEVKEPTTVVATNIDIELWKKHYDFKIYSWNGTFEFRGSHGFFDTYVDHFYQIKKNSTGGLRQIAKLHLNSLYGKFATNPDITGKHPTLKDNRVSLVMNEPETRDPVYTPMGVFITAYARKKTISAAQDNYETFAYADTDSLHLIGPTTPPDSLWVDPVELGAWRHESSFTKSVYIRAKQYAEEIGGKLDVHIAGMPRNVAATLTLEDMLHGGTWNGKLIPVRVPGGTVLKDTTFTLKID

SEQ ID NO: 21 - protein, 566 aa, synthetic construct
  source 1..566: organism (original language) = 合成构建体
MVRQSTIASPARGGVRRSHKKVPSFCADFETTTDEDDCRVWSWGIIQVGKLQNYVDGISLDGFMSHISERASHIYFHNLAFDGTFILDWLLKHGYRWTKENPGVKEFTSLISRMGKYYSITVVFETGFRVEFRDSFKKLPMSVSAIAKAFNLHDQKLEIDYEKPRPIGYIPTEQEKRYQRNDVAIVAQALEVQFAEKMTKLTAGSDSLATYKKMTGKLFIRRFPILSPEIDTEIRKAYRGGFTYADPRYAKKLNGKGSVYDVNSLYPSVMRYALLPYGEPIYSEGAPRTNRPLYIASITFTAKLKPNHIPCIQIKKNLSFNPTQYLEEVKEPTTVVATNIDIELWKKHYDFKIYSWNGTFEFRGSHGFFDTYVDHFYQIKKNSTGGLRQIAKLHLNSLYGKFATNPDITGKHPTLKDNRVSLVMNEPETRDPVYTPMGVFITAYARKKTISAAQDNYETFAYADTDSLHLIGPTTPPDSLWVDPVELGAWRHESSFTKSVYIRAKQYAEEIQGKLDVHIAGMPRNVAATLTLEDMLHGGTWNGKLIPVRVPGGTVLKDTTFTLKID

SEQ ID NO: 22 - protein, 566 aa, synthetic construct
  source 1..566: organism (original language) = 合成构建体
MVRQSTIASPARGGVRRSHKKVPSFCAQFETTTDEDDCRVWSWGIIQVGKLQNYVDGISLDGFMSHISERASHIYFHNLAIDGTFILDWLLKHGYRWTKENPGVKEFTSLISRMGKYYSITVVFETGFRVEFRDSFKKLPMSVSAIAKAFNLHDQKLEIDYEKPRPIGYIPTEQEKRYQRNDVAIVAQALEVQFAEKMTKLTAGSDSLATYKKMTGKLFIRRFPILSPEIDTEIRKAYRGGFTYADPRYAKKLNGKGSVYDVNSLYPSVMRTALLPYGEPIYSEGAPRTNRPLYIASITFTAKLKPNHIPCICIKKNLSFNPTQYLEEVKEPTTVVATNIDIELWKKHYDFKIYSWNGTFEFRGSHGFFDTYVDHFMEIKKNSTGGLRQIAKLHLNSLYGKFATNPDITGKHPTLKDNRVSLVMNEPETRDPVYTPMGVFITAYARKKTISAAQDNYETFAYADTDSLHLIGPTTPPDSLWVDPVELGAWRHESSFTKSVYIRAKQYAEEIGGKLRVHIAGMPRNVAATLTLEDMLHGGTWNGKLIPVRVPGGTVLKDTTFTLKID

SEQ ID NO: 23 - protein, 566 aa, synthetic construct
  source 1..566: organism (original language) = 合成构建体
MVRQSTIASPARGGVRRSHKKVPSFCADFETTTDEDDCRVWSWQIIQVGKLQNYVDGISLDGFMSHISERASHIYFHNLAVDGTFILDWLLKHGYRWTKENPGVKEFTSLISRMGKYYSITVVFETGFRVEFRDSFKKLPMSVSAIAKAFNLHDQKLEIDYEKPRPIGYIPTEQEKRYQRNDVAIVAQALEVQFAEKMTKLTAGSDSLATYKKMTGKLFIRRFPILSPEIDTEIRKAYRGGFTYADPRYAKKLNGKGSVYDVNSLYPSVMRTALLPYGEPIYSEGAPRTNRPLYIASITFTAKLKPNHIPCIQIKKNLSFNPTQYLEEVKEPTTVVATNIDIELWKKHYDFKIYSWNGTFEFRGSHGFFDTYVDHFMEIKKNSTGGLRQIAKLILNSLYGKFATNPDITGKHPTLKDNRVSLVMNEPETRDPVYTPMGVFITAYARKKTISAAQDNYETFAYADTDSLHLIGPTTPPDSLWVDPVELGAWRHESSFTKSVYLRAKQYAEEIGGKLDVHIAGMPRNVAATLTLEDMLHGGTWNGKLIPVRVPGGTVLKDTTFTLKID

SEQ ID NO: 24 - protein, 566 aa, synthetic construct
  source 1..566: organism (original language) = 合成构建体
MVRQSTIASPARGGVRRSHKKVPSFCADFETTTDEDDCRVWSWGIIQVGKLQNYVDGISLDGFMSHISERASHIYFHNLAIDGTFILDWLLKHGYRWTKENPGVKEFTSLISRMGKYYSITVVFETGFRVEFRDSFKKLPMSVSAIAKAFNLHDQKLEIDYEKPRPIGYIPTEQEKRYQRNDVAIVAQALEVQFAEKMTKLTAGSDSLATYKKMTGKLFIRRFPILSPEIDTEIRKAYRGGFTYADPRYAKKLNGKGSVYDVNSLYPSVMRTALLPYGEPIYSEGAPRTNRPLYIASITFTAKLKPNHIPCIQIKKNLSFNPTQYLEEVKEPTTVVATNIDIELWKKHYDFKIYSWNGTFEFRGSHGFFDDYVDHFMQIKKNSKGGLRQIAKLHLNSLYGKFATNPDITGKHPTLKDNRVSLVMNEPETRDPVYTPMGVFITAYARKKTISAAQDNYETFAYADTDSLHLIGPTTPPDSLWVDPVELGAWKHESSFTKSVYIRAKQYAEEIQGKLDVHIAGMPRNVAATLTLEDMLHGGTWNGKLIPVRVPGGTVLKDTTFTLKID

SEQ ID NO: 25 - protein, 566 aa, synthetic construct
  source 1..566: organism (original language) = 合成构建体
MVRQSTIASPARGGVRRSHKKVPSFCADFETTTDEDDCRVWSWGIIQVGKLQNYVDGISLDGFMSHISERASHIYFHNLAIDGTFILDWLLKHGYRWTKENPGVKEFTSLISRMGKYYSITVVFETGFRVEFRDSFKKLPMSVSAIAKAFNLHDQKLEIDYEKPRPIGYIPTEQEKRYQRNDVAIVAQALEVQFAEKMTKLTAGSDSLATYKKMTGKLFIRRFPILSPEIDTEIRKAYRGGFTYADPRYAKKLNGKGSVYDVNSLYPSVMRTALLPYGEPIYSEGAPRTNRPLYIASITFTAKLKPNHIPCIQIKKNLSFNPTQYLEEVKEPTTVVATNIDIELWKKHYDFKIYSWNGTFEFRGSHGFFDDYVDHFMQIKKNSKGGLRQIAKLHLNSLYGKFATNPDITGKHPTLKDNRVSLVMNEPETRDPVYTPMGVFITAYARKKTISAAQDNYETFAYADTDSLHLIGPTTPPDSLWVDPVELGAWKHESSFTKSVYIRAKQYAEEIDGKLRVHIAGMPRNVAATLTLEDMLHGGTWNGKLIPVRVPGGTVLKDTTFTLKID

SEQ ID NO: 26 - protein, 566 aa, synthetic construct
  source 1..566: organism (original language) = 合成构建体
MVRQSTIASPARGGVRRSHKKVPSFCADFETTTDEDDCRVWSWGIIQVGKLQNYVDGISLDGFMSHISERASHIYFHNLAFDGTFILDWLLKHGYRWTKENPGVKEFTSLISRMGRYYSITVVFETGFRVEFRDSFKKLPMSVSAIAKAFNLHDQKLEIDYEKPRPIGYIPTEQEKRYQRNDVAIVAQALEVQFAEKMTKLTAGSDSLATYKKMTGKLFIRRFPINSPEIDTEIRKAYRGGFTYADPRYAKKLNGKGSVYDVNSLYPSVMRTALLPYGEPIYSEGAPRTNRPLYIASITFTAKLKPNHIPCIYIKKNLSFNPTQYLEEVKEPTTVVATNIDIELWKKHYDFKIYSWNGTFEFRGSHGFFDTFVDHFMEIKKNSTGGLRQIAKLILNSLYGKFATNPDITGKHPTLKDNRVSLVMNEPETRDPVYTPMGVFITAYARKKTISAAQDNYETFAYADTDSLHLIGPTTPPDSLWVDPVELGAWKHESSFTKSVYIRAKQYAEEIGGKLDVHIAGMPRNVAATLTLEDMLHGGTWNGKLIPVRVPGGTVLKDTTFTLKID

SEQ ID NO: 27 - protein, 566 aa, synthetic construct
  source 1..566: organism (original language) = 合成构建体
MVRQSTIASPARGGVRRSHKKVPSFCADFETTTDEDDCRVWSWGIIQVGKLQNYVDGISLDGFMSHISERASHIYFHNLAFDGTFILDWLLKHGYRWTKENPGVKEFTSLISRMGRYYSITVVFETGFRVEFRDSFKKLPMSVSAIAKAFNLHDQKLEIDYEKPRPIGYIPTEQEKRYQRNDVAIVAQALEVQFAEKMTKLTAGSDSLATYKKMTGKLFIRRFPILSPEIDTEIRKAYRGGFTYADPRYAKKLNGKGSVYDVNSLYPSVMRTALLPYGEPIYSEGAPRTNRPLYIASITFTAKLKPNHIPCINIKKNNSFNPTQYLEEVKEPTTVVATNIDIELWKKHYDFKIYSWNGTFEFRGSHGFFDTFVDHFMEIKKNSTGGLRQIAKLILNSLYGKFATNPDITGKHPTLKDNRVSLVMNEPETRDPVYTPMGVFITAYARKKTISAAQDNYETFAYADTDSLHLIGPTTPPDSLWVDPVELGAWKHESSFTKSVYIRAKQYAEEIGGKLDVHIAGMPRNVAATLTLEDMLHGGTWNGKLIPVRVPGGTVLKDTTFTLKID

SEQ ID NO: 28 - protein, 566 aa, synthetic construct
  source 1..566: organism (original language) = 合成构建体
MVRQSTIASPARGGVRRSHKKVPSFCADFETTTDEDDCRVWSWGIIQVGKLQNYVDGISLDGFMSHISERASHIYFHNLAFDGTFILDWLLKHGYRWTKENPGVKEFTSLISRMGKYYSITVVFETGFRVEFRDSFKKLPMSVSAIAKAFNLHDQKLEIDLEKPRPIGYIPTEQEKRYQRNDVAIVAQALEVQFAEKMTKLTAGSDSLATYKKMTGKLFIRRFPILSPEIDTEIRKAYRGGFTYADPRYAKKLNGKGSVYDVNSAYPNVMRTALLPYGEPIYSEGAPRTNRPLYIASITFTAKLKPNHIPCIQIKKNLSFNPTQYLEEVKEPTTVVATNIDIELWKKHYDFKIYSWNGTFEFRGSHGFFDTYVDHFMEIKKNSKGGLRQIAKLHLNSTYGKFATNPDITGKHPTLKDNRVSLVMNEPETRDPVYTPMGVFITAYARKKTISAAQDNYETFAYADTDSLHLIGPTTPPDSLWVDPVELGAWKHESSFTKSVYIRAKQYAEEIGGKLDVHIAGMPRNVAATLTLEDMLHGGTWNGKLIPVRVPGGTVLKDTTFTLKID

SEQ ID NO: 29 - protein, 566 aa, synthetic construct
  source 1..566: organism (original language) = 合成构建体
MVRQSTIASPARGGVRRSHKKVPSFCADFETTTDEDDCRVWSWGIIQVGKLQNYVDGISLDGFMSHISERASHIYFHNLAIDGTFILDWLLKHGYRWTKENPGVKEFTSLISRMGKYYSITVVFETGFRVEFRDSFKKLPMSVSAIAKAFNLHDQKLEIDYEKPRPIGYIPTEQEKRYQRNDVAIVAQALEVQFAEKMTKLTAGSDSLATYKKMTGKLFIRRFPILSPEIDTEIRKAYRGGFTYADPRYAKKLNGKGSVYDVNSAYPSVMRTALLPYGEPIYSEGAPRTNRPLYIASITFTAKLKPNHIPCIQIKKNLSFNPTQYLEEVKEPTTVVATNIDIELWKKHYDFKIYSWNGTFEFRGSHGFFDTYVDHFMQIKKNSKGGLRQIAKLHLNSLYGKFATNPDITGKHPTLKDNRVSLVMNEPETRDPVYTPMGVFITAYARKKTISAAQDNYETFAYADTDSLHLIGPTTPPDSLWVDPVELGAWRHKSSFTKSVYLRAKQYAEEIGGKLDVHIAGMPRNVAATLTLEDMLHGGTWNGKLIPVRVPGGTVLKDTTFTLKID

SEQ ID NO: 30 - protein, 566 aa, synthetic construct
  source 1..566: organism (original language) = 合成构建体
MVRQSTIASPARGGVRRSHKKVPSFCADFETTTDEDDCRVWSWGIIQVGKLQNYVDGISLDGFMSHISERASHIYFHNLAIDGTFILDWLLKHGYRWTKENPGVKEFTSLISRMGKYYSITVVFETGFRVEFRDSFKKLPMSVSAIAKAFNLHDQKLEIDYEKPRPIGYIPTEQEKRYQRNDVAIVAQALEVQFAEKMTKLTAGSDSLATYKKMTGKLFIRRFPILSPEIDTEIRKAYRGGFTYADPRYAKKLNGKGSVYDVNSAYPSVMRTALLPYGEPIYSEGAPRTNRPLYIASITFTAKLKPNHIPCIQIKKNLSFNPTQYLEEVKEPTTVVATNIDIELWKKHYDFKIYSWNGTFEFRGSHGFFDTYVDHFMQIKKNSKGGLRRIAKLHLNSLYGKFATNPDITGKHPTLKDNRVSLVMNEPETRDPVYTPMGVFITAYARKKTISAAQDNYETFAYADTDSLHLIGPTTPPDSLWVDPVELGAWRHQSSFTKSVYIRAKQYAEEIGGKLRVHIAGMPRNVAATLTLEDMLHGGTWNGKLIPVRVPGGTVLKDTTFTLKID

SEQ ID NO: 31 - protein, 566 aa, synthetic construct
  source 1..566: organism (original language) = 合成构建体
MVRQSTIASPARGGVRRSHKKVPSFCADFETTTDEDDCRVWSWGIIQVGKLQNYVDGISLDGFMSHISERASHIYFHNLAIDGTFILDWLLKHGYRWTKENPGVKEFTSLISRMGKYYSITVVFETGFRVEFRDSFKKLPMSVSAIAKAFNLHDQKLEIDYEKPRPIGYIPTEQEKRYQRNDVAIVAQALEVQFAEKMTKLTAGSDSLATYKKMTGKLFIRRFPILSPEIDTEIRKAYRGGFTYADPRYAKKLNGKGSVYDVNSLYPSVMRYALLPYGEPIYSEGAPRTNRPLYIASITFTAKLKPNHIPCIQIKKNLSFNPTQYLEEVKEPTTVVATNIDIELWKKHYDFKIYSWNGTFEFRGSHGFFDTYVDHFYQIKKNSTGGLRQIAKLHLNSLYGKFATNPDITGKHPTLKDNRVSLVMNEPETRDPVYTPMGVFITAYARKKTISAAQDNYETFAYADTDSLHLIGPTTPPDSLWVDPVELGAWRHESSFTKSVYIRAKQYAEEIQGKLDVHIAGMPRNVAATLTLEDMLHGGTWNGKLIPVRVPGGTVLKDTTFTLKID

SEQ ID NO: 32 - protein, 566 aa, synthetic construct
  source 1..566: organism (original language) = 合成构建体
MVRQSTIASPARGGVRRSHKKVPSFCADFETTTDEDDCRVWSWGIIQVGKLQNYVDGISLDGFMSHISERASHIYFHNLAVDGTFILDWLLKHGYRWTKENPGVKEFTSLISRMGKYYSITVVFETGFRVEFRDSFKKLPMSVSAIAKAFNLHDQKLEIDYEKPRPIGYIPTEQEKRYQRNDVAIVAQALEVQFAEKMTKLTAGSDSLATYKKMTGKLFIRRFPILSPEIDTEIRKAYRGGFTYADPRYAKKLNGKGSVYDVNSLYPSVMRYALLPYGEPIYSEGAPRTNRPLYIASITFTAKLKPNHIPCIQIKKNLSFNPTQYLEEVKEPTTVVATNIDIELWKKHYDFKIYSWNGTFEFRGSHGFFDTYVDHFYQIKKNSTGGLRQIAKLHLNSLYGKFATNPDITGKHPTLKDNRVSLVMNEPETRDPVYTPMGVFITAYARKKTISAAQDNYETFAYADTDSLHLIGPTTPPDSLWVDPVELGAWRHESSFTKSVYIRAKQYAEEIQGKLDVHIAGMPRNVAATLTLEDMLHGGTWNGKLIPVRVPGGTVLKDTTFTLKID

SEQ ID NO: 33 - protein, 566 aa, synthetic construct
  source 1..566: organism (original language) = 合成构建体
MVRQSTIASPARGGVRRSHKKVPSFCADFETTTDEDDCRVWSWGIIQVGKLQNYVDGISLDGFMSHISERASHIYFHNLAIDGTFILDWLLKHGYRWTKENPGVKEFTSLISRMGKYYSITVVFETGFRVEFRDSFKKLPMSVSAIAKAFNLHDQKLEIDYEKPRPIGYIPTEQEKRYQRNDVAIVAQALEVQFAEKMTKLTAGSDSLATYKKMTGKLFIRRFPILSPEIDTEIRKAYRGGFTYADPRYAKKLNGKGSVYDVNSLYPSVMRYALLPYGEPIYSEGAPRTNRPLYIASITFTAKLKPNHIPCIQIKKNLSFNPTQYLEEVKEPTTVVATNIDIELWKKHYDFKIYSWNGTFEFRGSHGFFDTYVDHFYQIKKNSTGGLRQIAKLHLNSLYGKFATNPDITGKHPTLKDNRVSLVMNEPETRDPVYTPMGVFITAYARKKTISAAQDNYETFAYADTDSLHLIGPTTPPDSLWVDPVELGAWRHESSFTKSVYLRAKQYAEEIQGKLDVHIAGMPRNVAATLTLEDMLHGGTWNGKLIPVRVPGGTVLKDTTFTLKID

SEQ ID NO: 34 - protein, 566 aa, synthetic construct
  source 1..566: organism (original language) = 合成构建体
MVRQSTIASPARGGVRRSHKKVPSFCADFETTTDEDDCRVWSWQIIQVGKLQNYVDGISLDGFMSHISERASHIYFHNLAFDGTFILDWLLKHGYRWTKENPGVKEFTSLISRMGKYYSITVVFETGFRVEFRDSFKKLPMSVSAIAKAFNLHDQKLEIDYEKPRPIGYIPTEQEKRYQRNDVAIVAQALEVQFAEKMTKLTAGSDSLATYKKMTGKLFIRRFPILSPEIDTEIRKAYRGGFTYADPRYAKKLNGKGSVYDVNSLYPSVMRSALLPYGEPIYSEGAPRTNRPLYIASITFTAKLKPNHIPCIQIKKNLSFNPTQYLEEVKEPTTVVATNIDIELWKKHYDFKIYSWNGTFEFRGSHGFFDTYVDHFMDIKKNSTGGLRQIAKLHLNSLYGKFATNPDITGKHPTLKDNRVSLVMNEPETRDPVYTPMGVFITAYARKKTISAAQDNYETFAYADTDSLHLIGPTTPPDSLWVDPVELGAWKHKSSFTKSVYIRAKQYAEEIQGKLRVHIAGMPRNVAATLTLEDMLHGGTWNGKLIPVRVPGGTVLKDTTFTLKID

SEQ ID NO: 35 - protein, 566 aa, synthetic construct
  source 1..566: organism (original language) = 合成构建体
MVRQSTIASPARGGVRRSHKKVPSFCADFETTTDEDDCRVWSWGIIQVGKLQNYVDGISLDGFMSHISERASHIYFHNLAFDGTFILDWLLKHGYRWTKENPGVKEFTSLISRMGRYYSITVVFETGFRVEFRDSFKKLPMSVSAIAKAFNLHDQKLEIDYEKPRPIGYIPTEQEKRYQRNDVAIVAQALEVQFAEKMTKLTAGSDSLATYKKMTGKLFIRRFPILSPEIDTEIRKAYRGGFTYADPRYAKKLNGKGSVYDVNSLYPSVMRTALLPYGEPIYSEGAPRTNRPLYIASITFTAKLKPNHIPCINIKKNNSFNPTQYLEEVKEPTTVVATNIDIELWKKHYDFKIYSWNGTFEFRGSHGFFDTFVDHFMEIKKNSTGGLRQIAKLILNSLYGKFATNPDITGKHPTLKDNRVSLVMNEPETRDPVYTPMGVFITAYARKKTISAAQDNYETFAYADTDSLHLIGPTTPPDSLWVDPVELGAWKHESSFTKSVYLRAKQYAEEIGGKLDVHIAGMPRNVAATLTLEDMLHGGTWNGKLIPVRVPGGTVLKDTTFTLKID

SEQ ID NO: 36 - protein, 566 aa, synthetic construct
  source 1..566: organism (original language) = 合成构建体
MVRQSTIASPARGGVRRSHKKVPSFCADFETTTDEDDCRVWSWGIIQVGKLQNYVDGISLDGFMSHISERASHIYFHNLAVDGTFILDWLLKHGYRWTKENPGVKEFTSLISRMGRYYSITVVFETGFRVEFRDSFKKLPMSVSAIAKAFNLHDQKLEIDYEKPRPIGYIPTEQEKRYQRNDVAIVAQALEVQFAEKMTKLTAGSDSLATYKKMTGKLFIRRFPILSPEIDTEIRKAYRGGFTYADPRYAKKLNGKGSVYDVNSLYPSVMRTALLPYGEPIYSEGAPRTNRPLYIASITFTAKLKPNHIPCINIKKNNSFNPTQYLEEVKEPTTVVATNIDIELWKKHYDFKIYSWNGTFEFRGSHGFFDTFVDHFMEIKKNSTGGLRQIAKLILNSLYGKFATNPDITGKHPTLKDNRVSLVMNEPETRDPVYTPMGVFITAYARKKTISAAQDNYETFAYADTDSLHLIGPTTPPDSLWVDPVELGAWKHESSFTKSVYIRAKQYAEEIGGKLDVHIAGMPRNVAATLTLEDMLHGGTWNGKLIPVRVPGGTVLKDTTFTLKID

SEQ ID NO: 37 - DNA, 97 bp, synthetic construct
  source 1..97: mol_type = other DNA; organism (original language) = 合成构建体
cctaccgtatcgttttaccagtcagtcagtcagtcagtcagtcagtcagtcagtcagctaagcacctgtcttcgcttttgcgaagacaggtgcttag

SEQ ID NO: 38 - DNA, 22 bp, synthetic construct
  source 1..22: mol_type = other DNA; organism (original language) = 合成构建体
gtccgtaaaacgatacggtagg

SEQ ID NO: 39 - DNA, 88 bp, synthetic construct
  source 1..88: mol_type = other DNA; organism (original language) = 合成构建体
gcgcctttccagacgcttaccaagagcaactacacgaattctcgattaggttactgcgattagcacaagcgctgtcaccctgtatcgc

SEQ ID NO: 40 - DNA, 22 bp, synthetic construct
  source 1..22: mol_type = other DNA; organism (original language) = 合成构建体
ggaaaggcgcgcgatacagggt